European Patent Application EP 4 421 180 A2, published August 28, 2024. Title: COMPOSITIONS COMPRISING NKG2D, CXCR2, AND DAP10/DAP12 FUSION POLYPEPTIDES AND METHODS OF USE THEREOF. Applicant: KING'S COLLEGE LONDON. Application EP. The sequence listing filed with the application follows.

SEQUENCE LISTING (115 sequences)

SEQ ID NO: 1 - protein, 93 aa, Homo sapiens
MIHLGHILFLLLLPVAAAQTTPGERSSLPAFYPGTSGSCSGCGSLSLPLLAGLVAADAVASLLIVGAVFLCARPRRSPAQEDGKVYINMPGRG

SEQ ID NO: 2 - protein, 75 aa, Homo sapiens
QTTPGERSSLPAFYPGTSGSCSGCGSLSLPLLAGLVAADAVASLLIVGAVFLCARPRRSPAQEDGKVYINMPGRG

SEQ ID NO: 3 - protein, 51 aa, Homo sapiens
QTTPGERSSLPAFYPGTSGSCSGCGSLSLPLLAGLVAADAVASLLIVGAVF

SEQ ID NO: 4 - protein, 71 aa, Homo sapiens
MIHLGHILFLLLLPVAAAQTTPGERSSLPAFYPGTSGSCSGCGSLSLPLLAGLVAADAVASLLIVGAVFLC

SEQ ID NO: 5 - protein, 53 aa, Homo sapiens
QTTPGERSSLPAFYPGTSGSCSGCGSLSLPLLAGLVAADAVASLLIVGAVFLC

SEQ ID NO: 6 - protein, 24 aa, Homo sapiens
LCARPRRSPAQEDGKVYINMPGRG

SEQ ID NO: 7 - protein, 45 aa, Homo sapiens
LLAGLVAADAVASLLIVGAVFLCARPRRSPAQEDGKVYINMPGRG

SEQ ID NO: 8 - protein, 21 aa, Homo sapiens
LLAGLVAADAVASLLIVGAVF

SEQ ID NO: 9 - protein, 113 aa, Homo sapiens
MGGLEPCSRLLLLPLLLAVSGLRPVQAQAQSDCSCSTVSPGVLAGIVMGDLVLTVLIALAVYFLGRLVPRGRGAAEAATRKQRITETESPYQELQGQRSDVYSDLNTQRPYYK

SEQ ID NO: 10 - protein, 92 aa, Homo sapiens
LRPVQAQAQSDCSCSTVSPGVLAGIVMGDLVLTVLIALAVYFLGRLVPRGRGAAEAATRKQRITETESPYQELQGQRSDVYSDLNTQRPYYK

SEQ ID NO: 11 - protein, 52 aa, Homo sapiens
YFLGRLVPRGRGAAEAATRKQRITETESPYQELQGQRSDVYSDLNTQRPYYK

SEQ ID NO: 12 - protein, 21 aa, Homo sapiens
GVLAGIVMGDLVLTVLIALAV

SEQ ID NO: 13 - protein, 40 aa, Homo sapiens
LRPVQAQAQSDCSCSTVSPGVLAGIVMGDLVLTVLIALAV

SEQ ID NO: 14 - protein, 216 aa, Homo sapiens
MGWIRGRRSRHSWEMSEFHNYNLDLKKSDFSTRWQKQRCPVVKSKCRENASPFFFCCFIAVAMGIRFIIMVAIWSAVFLNSLFNQEVQIPLTESYCGPCPKNWICYKNNCYQFFDESKNWYESQASCMSQNASLLKVYSKEDQDLLKLVKSYHWMGLVHIPTNGSWQWEDGSILSPNLLTIIEMQKGDCALYASSFKGYIENCSTPNTYICMQRTV

SEQ ID NO: 15 - protein, 144 aa, Homo sapiens
IWSAVFLNSLFNQEVQIPLTESYCGPCPKNWICYKNNCYQFFDESKNWYESQASCMSQNASLLKVYSKEDQDLLKLVKSYHWMGLVHIPTNGSWQWEDGSILSPNLLTIIEMQKGDCALYASSFKGYIENCSTPNTYICMQRTV

SEQ ID NO: 16 - protein, 135 aa, Homo sapiens
LFNQEVQIPLTESYCGPCPKNWICYKNNCYQFFDESKNWYESQASCMSQNASLLKVYSKEDQDLLKLVKSYHWMGLVHIPTNGSWQWEDGSILSPNLLTIIEMQKGDCALYASSFKGYIENCSTPNTYICMQRTV

SEQ ID NO: 17 - protein, 165 aa, Homo sapiens
PFFFCCFIAVAMGIRFIIMVAIWSAVFLNSLFNQEVQIPLTESYCGPCPKNWICYKNNCYQFFDESKNWYESQASCMSQNASLLKVYSKEDQDLLKLVKSYHWMGLVHIPTNGSWQWEDGSILSPNLLTIIEMQKGDCALYASSFKGYIENCSTPNTYICMQRTV

SEQ ID NO: 18 - skipped

SEQ ID NO: 19 - protein, 5 aa, synthetic construct
GSGGG

SEQ ID NO: 20 - protein, 4 aa, synthetic construct
GSGG

SEQ ID NO: 21 - protein, 4 aa, synthetic construct
SGGG

SEQ ID NO: 22 - protein, 5 aa, synthetic construct
GGGGS

SEQ ID NO: 23 - protein, 20 aa, synthetic construct
GGGGSGGGGSGGGGSGGGGS

SEQ ID NO: 24 - protein, 15 aa, synthetic construct
GGGGSGGGGSGGGGS

SEQ ID NO: 25 - protein, 5 aa, synthetic construct
GPPGS

SEQ ID NO: 26 - protein, 4 aa, synthetic construct
GGGS

SEQ ID NO: 27 - protein, 5 aa, synthetic construct
GGGGS

SEQ ID NO: 28-29 - skipped (2 entries)

SEQ ID NO: 30 - protein, 5 aa, synthetic construct
SGGGG

SEQ ID NO: 31 - protein, 4 aa, synthetic construct
SGGG

SEQ ID NO: 32 - skipped

SEQ ID NO: 33 - protein, 4 aa, synthetic construct
SGSG

SEQ ID NO: 34 - skipped

SEQ ID NO: 35 - protein, 5 aa, synthetic construct
GGGGA

SEQ ID NO: 36 - protein, 4 aa, synthetic construct
GGGA

SEQ ID NO: 37 - protein, 5 aa, synthetic construct
EAAAK

SEQ ID NO: 38 - protein, 4 aa, synthetic construct
RRKR

SEQ ID NO: 39 - protein, 19 aa, synthetic construct
ATNFSLLKQAGDVEENPGP

SEQ ID NO: 40 - protein, 18 aa, synthetic construct
EGRGSLLTCGDVEENPGP

SEQ ID NO: 41 - protein, 23 aa, synthetic construct
SGSGATNFSLLKQAGDVEENPGP

SEQ ID NO: 42 - protein, 22 aa, synthetic construct
SGSGEGRGSLLTCGDVEENPGP

SEQ ID NO: 43 - protein, 27 aa, synthetic construct
RRKRSGSGATNFSLLKQAGDVEENPGP

SEQ ID NO: 44 - protein, 26 aa, synthetic construct
RRKRSGSGEGRGSLLTCGDVEENPGP

SEQ ID NO: 45 - protein, 22 aa, synthetic construct
VKQTLNFDLLKLAGDVESNPGP

SEQ ID NO: 46 - protein, 20 aa, synthetic construct
QCTNYALLKLAGDVESNPGP

SEQ ID NO: 47 - protein, 6 aa, synthetic construct
HHHHHH

SEQ ID NO: 48 - protein, 8 aa, synthetic construct
DYKDDDDK

SEQ ID NO: 49 - protein, 15 aa, synthetic construct
GLNDIFEAQKIEWHE

SEQ ID NO: 50 - protein, 14 aa, synthetic construct
GKPIPNPLLGLDST

SEQ ID NO: 51 - protein, 9 aa, synthetic construct
IPNPLLGLD

SEQ ID NO: 52 - protein, 10 aa, synthetic construct
EQKLISEEDL

SEQ ID NO: 53 - protein, 31 aa, synthetic construct
GLNDIFEAQKIEWHEGGHHHHHHDYKDDDDK

SEQ ID NO: 54 - protein, 31 aa, synthetic construct
DYKDDDDKHHHHHHGGGLNDIFEAQKIEWHE

SEQ ID NO: 55 - protein, 21 aa, Homo sapiens
MALPVTALLLPLALLLHAARP

SEQ ID NO: 56 - protein, 42 aa, Homo sapiens
KRGRKKLLYIFKQPFMRPVQTTQEEDGCSCRFPEEEEGGCEL

SEQ ID NO: 57 - protein, 48 aa, Homo sapiens
QRRKYRSNKGESPVEPAEPCHYSCPREEEGSTIPIQEDYRKPEPACSP

SEQ ID NO: 58 - protein, 12 aa, Homo sapiens
EPKSCDKTHTCP

SEQ ID NO: 59 - protein, 45 aa, Homo sapiens
TTTPAPRPPTPAPTIASQPLSLRPEACRPAAGGAVHTRGLDFACD

SEQ ID NO: 60 - protein, 145 aa, synthetic construct
MIHLGHILFLLLLPVAAAQTTPGERSSLPAFYPGTSGSCSGCGSLSLPLLAGLVAADAVASLLIVGAVFLCARPRRSPAQEDGKVYINMPGRGYFLGRLVPRGRGAAEAATRKQRITETESPYQELQGQRSDVYSDLNTQRPYYK

SEQ ID NO: 61 - protein, 132 aa, synthetic construct
MALPVTALLLPLALLLHAARPDYKDDDDKQTTPGERSSLPAFYPGTSGSCSGCGSLSLPLLAGLVAADAVASLLIVGAVFYFLGRLVPRGRGAAEAATRKQRITETESPYQELQGQRSDVYSDLNTQRPYYK

SEQ ID NO: 62 - protein, 138 aa, synthetic construct
MALPVTALLLPLALLLHAARPDYKDDDDKEPKSCDKTHTCPLLAGLVAADAVASLLIVGAVFLCARPRRSPAQEDGKVYINMPGRGYFLGRLVPRGRGAAEAATRKQRITETESPYQELQGQRSDVYSDLNTQRPYYK

SEQ ID NO: 63 - protein, 171 aa, synthetic construct
MALPVTALLLPLALLLHAARPDYKDDDDKTTTPAPRPPTPAPTIASQPLSLRPEACRPAAGGAVHTRGLDFACDLLAGLVAADAVASLLIVGAVFLCARPRRSPAQEDGKVYINMPGRGYFLGRLVPRGRGAAEAATRKQRITETESPYQELQGQRSDVYSDLNTQRPYYK

SEQ ID NO: 64 - protein, 388 aa, synthetic construct
MIHLGHILFLLLLPVAAAQTTPGERSSLPAFYPGTSGSCSGCGSLSLPLLAGLVAADAVASLLIVGAVFLCARPRRSPAQEDGKVYINMPGRGYFLGRLVPRGRGAAEAATRKQRITETESPYQELQGQRSDVYSDLNTQRPYYKRRKRSGSGATNFSLLKQAGDVEENPGPMGWIRGRRSRHSWEMSEFHNYNLDLKKSDFSTRWQKQRCPVVKSKCRENASPFFFCCFIAVAMGIRFIIMVAIWSAVFLNSLFNQEVQIPLTESYCGPCPKNWICYKNNCYQFFDESKNWYESQASCMSQNASLLKVYSKEDQDLLKLVKSYHWMGLVHIPTNGSWQWEDGSILSPNLLTIIEMQKGDCALYASSFKGYIENCSTPNTYICMQRTV

SEQ ID NO: 65 - protein, 494 aa, synthetic construct
MALPVTALLLPLALLLHAARPDYKDDDDKQTTPGERSSLPAFYPGTSGSCSGCGSLSLPLLAGLVAADAVASLLIVGAVFYFLGRLVPRGRGAAEAATRKQRITETESPYQELQGQRSDVYSDLNTQRPYYKRRKRSGSGEGRGSLLTCGDVEENPGPMIHLGHILFLLLLPVAAAQTTPGERSSLPAFYPGTSGSCSGCGSLSLPLLAGLVAADAVASLLIVGAVFLCARPRRSPAQEDGKVYINMPGRGRRKRSGSGATNFSLLKQAGDVEENPGPMGWIRGRRSRHSWEMSEFHNYNLDLKKSDFSTRWQKQRCPVVKSKCRENASPFFFCCFIAVAMGIRFIIMVAIWSAVFLNSLFNQEVQIPLTESYCGPCPKNWICYKNNCYQFFDESKNWYESQASCMSQNASLLKVYSKEDQDLLKLVKSYHWMGLVHIPTNGSWQWEDGSILSPNLLTIIEMQKGDCALYASSFKGYIENCSTPNTYICMQRTV

SEQ ID NO: 66 - protein, 527 aa, synthetic construct
MIHLGHILFLLLLPVAAAQTTPGERSSLPAFYPGTSGSCSGCGSLSLPLLAGLVAADAVASLLIVGAVFLCARPRRSPAQEDGKVYINMPGRGYFLGRLVPRGRGAAEAATRKQRITETESPYQELQGQRSDVYSDLNTQRPYYKRRKRSGSGATNFSLLKQAGDVEENPGPMGWIRGRRSRHSWEMSEFHNYNLDLKKSDFSTRWQKQRCPVVKSKCRENASPFFFCCFIAVAMGIRFIIMVAIWSAVFLNSLFNQEVQIPLTESYCGPCPKNWICYKNNCYQFFDESKNWYESQASCMSQNASLLKVYSKEDQDLLKLVKSYHWMGLVHIPTNGSWQWEDGSILSPNLLTIIEMQKGDCALYASSFKGYIENCSTPNTYICMQRTVRRKRSGSGEGRGSLLTCGDVEENPGPMIHLGHILFLLLLPVAAAQTTPGERSSLPAFYPGTSGSCSGCGSLSLPLLAGLVAADAVASLLIVGAVFLCKRGRKKLLYIFKQPFMRPVQTTQEEDGCSCRFPEEEEGGCEL

SEQ ID NO: 67 - protein, 538 aa, synthetic construct
MIHLGHILFLLLLPVAAAQTTPGERSSLPAFYPGTSGSCSGCGSLSLPLLAGLVAADAVASLLIVGAVFLCARPRRSPAQEDGKVYINMPGRGYFLGRLVPRGRGAAEAATRKQRITETESPYQELQGQRSDVYSDLNTQRPYYKRRKRSGSGATNFSLLKQAGDVEENPGPMGWIRGRRSRHSWEMSEFHNYNLDLKKSDFSTRWQKQRCPVVKSKCRENASPFFFCCFIAVAMGIRFIIMVAIWSAVFLNSLFNQEVQIPLTESYCGPCPKNWICYKNNCYQFFDESKNWYESQASCMSQNASLLKVYSKEDQDLLKLVKSYHWMGLVHIPTNGSWQWEDGSILSPNLLTIIEMQKGDCALYASSFKGYIENCSTPNTYICMQRTVRRKRSGSGEGRGSLLTCGDVEENPGPMALPVTALLLPLALLLHAARPDYKDDDDKQTTPGERSSLPAFYPGTSGSCSGCGSLSLPLLAGLVAADAVASLLIVGAVFLCKRGRKKLLYIFKQPFMRPVQTTQEEDGCSCRFPEEEEGGCEL

SEQ ID NO: 68 - protein, 533 aa, synthetic construct
MIHLGHILFLLLLPVAAAQTTPGERSSLPAFYPGTSGSCSGCGSLSLPLLAGLVAADAVASLLIVGAVFLCARPRRSPAQEDGKVYINMPGRGYFLGRLVPRGRGAAEAATRKQRITETESPYQELQGQRSDVYSDLNTQRPYYKRRKRSGSGATNFSLLKQAGDVEENPGPMGWIRGRRSRHSWEMSEFHNYNLDLKKSDFSTRWQKQRCPVVKSKCRENASPFFFCCFIAVAMGIRFIIMVAIWSAVFLNSLFNQEVQIPLTESYCGPCPKNWICYKNNCYQFFDESKNWYESQASCMSQNASLLKVYSKEDQDLLKLVKSYHWMGLVHIPTNGSWQWEDGSILSPNLLTIIEMQKGDCALYASSFKGYIENCSTPNTYICMQRTVRRKRSGSGEGRGSLLTCGDVEENPGPMIHLGHILFLLLLPVAAAQTTPGERSSLPAFYPGTSGSCSGCGSLSLPLLAGLVAADAVASLLIVGAVFLCQRRKYRSNKGESPVEPAEPCHYSCPREEEGSTIPIQEDYRKPEPACSP

SEQ ID NO: 69 - protein, 544 aa, synthetic construct
MIHLGHILFLLLLPVAAAQTTPGERSSLPAFYPGTSGSCSGCGSLSLPLLAGLVAADAVASLLIVGAVFLCARPRRSPAQEDGKVYINMPGRGYFLGRLVPRGRGAAEAATRKQRITETESPYQELQGQRSDVYSDLNTQRPYYKRRKRSGSGATNFSLLKQAGDVEENPGPMGWIRGRRSRHSWEMSEFHNYNLDLKKSDFSTRWQKQRCPVVKSKCRENASPFFFCCFIAVAMGIRFIIMVAIWSAVFLNSLFNQEVQIPLTESYCGPCPKNWICYKNNCYQFFDESKNWYESQASCMSQNASLLKVYSKEDQDLLKLVKSYHWMGLVHIPTNGSWQWEDGSILSPNLLTIIEMQKGDCALYASSFKGYIENCSTPNTYICMQRTVRRKRSGSGEGRGSLLTCGDVEENPGPMALPVTALLLPLALLLHAARPDYKDDDDKQTTPGERSSLPAFYPGTSGSCSGCGSLSLPLLAGLVAADAVASLLIVGAVFLCQRRKYRSNKGESPVEPAEPCHYSCPREEEGSTIPIQEDYRKPEPACSP

SEQ ID NO: 70 - DNA, 435 bp, synthetic construct
  source 1..435: mol_type = other DNA
atgatccacctgggccacatcctgttcctgctgctgctgcccgtggccgctgcccagaccacccctggcgagcggagcagcctgcctgccttctaccctggcaccagcggcagctgcagcggctgcggcagcctgagcctgcccctgctggccggcctggtggccgccgacgccgtggccagcctgctgatcgtgggcgccgtgttcctgtgcgccaggcccaggcggagccctgcccaggaggacggcaaggtgtacatcaacatgcccggccggggctacttcctgggcaggctggtgcccaggggcaggggcgctgccgaggctgccacccggaagcagcggatcaccgagaccgagagcccctaccaggagctgcagggccagcggagcgacgtgtacagcgacctgaacacccagaggccctactacaag

SEQ ID NO: 71 - DNA, 396 bp, synthetic construct
  source 1..396: mol_type = other DNA
atggctctgcctgtgacagctctgctgctgcctctggctctgctgctgcacgccgctagacccgattataaggacgacgacgacaagcagaccacccctggcgagcggagcagcctgcctgccttctaccctggcaccagcggcagctgcagcggctgcggcagcctgagcctgcccctgctggctggcctggtggccgccgacgccgtggccagcctgctgatcgtgggcgccgtgttctacttcctgggcaggctggtgcccaggggcaggggcgctgccgaggctgccacccggaagcagcggatcaccgagaccgagagcccctaccaggagctgcagggccagcggagcgacgtgtacagcgacctgaacacccagaggccctactacaag

SEQ ID NO: 72 - DNA, 414 bp, synthetic construct
  source 1..414: mol_type = other DNA
atggctctgcctgtgacagctctgctgctgcctctggctctgctgctgcacgccgctagacccgattataaggacgacgacgacaaggagcccaagagctgcgacaagacacacacatgccctcttctggccggcctggtggccgccgacgccgtggccagcctgctgatcgtgggcgccgtgttcctgtgcgccaggcccaggcggagccctgcccaggaggacggcaaggtgtacatcaacatgcccggccggggctacttcctgggcaggctggtgcccaggggcaggggcgctgccgaggctgccacccggaagcagcggatcaccgagaccgagagcccctaccaggagctgcagggccagcggagcgacgtgtacagcgacctgaacacccagaggccctactacaag

SEQ ID NO: 73 - DNA, 513 bp, synthetic construct
  source 1..513: mol_type = other DNA
atggctctgcctgtgacagctctgctgctgcctctggctctgctgctgcacgccgctagacccgattataaggacgacgacgacaagaccacaacacctgctcctagacctcccacccctgctcccaccatcgccagccagcccctgagcctgagacccgaggcctgcagacccgctgctggcggcgctgtgcataccagaggcctggatttcgcctgcgaccttctggccggcctggtggccgccgacgccgtggccagcctgctgatcgtgggcgccgtgttcctgtgcgccaggcccaggcggagccctgcccaggaggacggcaaggtgtacatcaacatgcccggccggggctacttcctgggcaggctggtgcccaggggcaggggcgctgccgaggctgccacccggaagcagcggatcaccgagaccgagagcccctaccaggagctgcagggccagcggagcgacgtgtacagcgacctgaacacccagaggccctactacaag

SEQ ID NO: 74 - DNA, 1164 bp, synthetic construct
  source 1..1164: mol_type = other DNA
atgatccacctgggccacatcctgttcctgctgctgctgcccgtggccgctgcccagaccacccctggcgagcggagcagcctgcctgccttctaccctggcaccagcggcagctgcagcggctgcggcagcctgagcctgcccctgctggccggcctggtggccgccgacgccgtggccagcctgctgatcgtgggcgccgtgttcctgtgcgccaggcccaggcggagccctgcccaggaggacggcaaggtgtacatcaacatgcccggccggggctacttcctgggcaggctggtgcccaggggcaggggcgctgccgaggctgccacccggaagcagcggatcaccgagaccgagagcccctaccaggagctgcagggccagcggagcgacgtgtacagcgacctgaacacccagaggccctactacaagaggcggaaaaggtctgggagtggggctaccaatttctctctcctcaagcaagccggagacgttgaggaaaaccctggacccatgggctggatccggggacggaggagccggcacagctgggagatgagcgagttccacaactacaacctggacctgaagaagagcgacttcagcacccggtggcagaagcagcggtgccccgtggtgaagagcaagtgccgggagaacgccagccccttcttcttctgctgcttcatcgccgtggctatgggcatccggttcatcatcatggtggccatctggagcgccgtgttcctgaacagcctgttcaaccaggaggtgcagatccccctgaccgagagctactgcggcccctgccccaagaactggatctgctacaagaacaactgctaccagttcttcgacgagagcaagaactggtacgagagccaggccagctgcatgagccagaacgccagcctgctgaaggtgtacagcaaggaggaccaggacctgctgaagctggtgaagagctaccactggatgggcctggtgcacatccccaccaacggcagctggcagtgggaggacggcagcatcctgagccccaacctgctgaccatcatcgagatgcagaagggcgactgcgccctgtacgccagcagcttcaagggctacatcgagaactgcagcacccccaacacctacatctgcatgcagcggaccgtg

SEQ ID NO: 75 - DNA, 1482 bp, synthetic construct
  source 1..1482: mol_type = other DNA
atggctctgcctgtgacagctctgctgctgcctctggctctgctgctgcacgccgctagacccgattataaggacgacgacgacaagcagaccacccctggcgagcggagcagcctgcctgccttctaccctggcaccagcggcagctgcagcggctgcggcagcctgagcctgcccctgctggctggcctggtggccgccgacgccgtggccagcctgctgatcgtgggcgccgtgttctacttcctgggcaggctggtgcccaggggcaggggcgctgccgaggctgccacccggaagcagcggatcaccgagaccgagagcccctaccaggagctgcagggccagcggagcgacgtgtacagcgacctgaacacccagaggccctactacaagcggagaaagcgctccggctccggcgagggccgcggcagcctgctgacctgcggcgacgtggaagagaaccccggacccatgatccacctgggccacatcctgttcctgctgctgctgcccgtggccgctgcccaaacaacacccggcgagagatcctccttgcccgctttctatcccggaacatccggaagctgttccggatgtggatccctttctttgcctttgcttgctggattggtcgcagctgacgctgtcgcttccctccttattgtcggagctgtcttcctgtgcgccaggcccaggcggagccctgcccaggaggacggcaaggtgtacatcaacatgcccggccggggcaggcggaagcgctccgggagtggggctaccaatttctctctcctcaagcaagccggagacgttgaggaaaaccctggacccatgggctggatccggggacggaggagccggcacagctgggagatgagcgagttccacaactacaacctggacctgaagaagagcgacttcagcacccggtggcagaagcagcggtgccccgtggtgaagagcaagtgccgggagaacgccagccccttcttcttctgctgcttcatcgccgtggctatgggcatccggttcatcatcatggtggccatctggagcgccgtgttcctgaacagcctgttcaaccaggaggtgcagatccccctgaccgagagctactgcggcccctgccccaagaactggatctgctacaagaacaactgctaccagttcttcgacgagagcaagaactggtacgagagccaggccagctgcatgagccagaacgccagcctgctgaaggtgtacagcaaggaggaccaggacctgctgaagctggtgaagagctaccactggatgggcctggtgcacatccccaccaacggcagctggcagtgggaggacggcagcatcctgagccccaacctgctgaccatcatcgagatgcagaagggcgactgcgccctgtacgccagcagcttcaagggctacatcgagaactgcagcacccccaacacctacatctgcatgcagcggaccgtg

SEQ ID NO: 76 - DNA, 1581 bp, synthetic construct
  source 1..1581: mol_type = other DNA
atgatccacctgggccacatcctgttcctgctgctgctgcccgtggccgctgcccagaccacccctggcgagcggagcagcctgcctgccttctaccctggcaccagcggcagctgcagcggctgcggcagcctgagcctgcccctgctggccggcctggtggccgccgacgccgtggccagcctgctgatcgtgggcgccgtgttcctgtgcgccaggcccaggcggagccctgcccaggaggacggcaaggtgtacatcaacatgcccggccggggctacttcctgggcaggctggtgcccaggggcaggggcgctgccgaggctgccacccggaagcagcggatcaccgagaccgagagcccctaccaggagctgcagggccagcggagcgacgtgtacagcgacctgaacacccagaggccctactacaagaggcggaaaaggtctgggagtggggctaccaatttctctctcctcaagcaagccggagacgttgaggaaaaccctggacccatgggctggatccggggacggaggagccggcacagctgggagatgagcgagttccacaactacaacctggacctgaagaagagcgacttcagcacccggtggcagaagcagcggtgccccgtggtgaagagcaagtgccgggagaacgccagccccttcttcttctgctgcttcatcgccgtggctatgggcatccggttcatcatcatggtggccatctggagcgccgtgttcctgaacagcctgttcaaccaggaggtgcagatccccctgaccgagagctactgcggcccctgccccaagaactggatctgctacaagaacaactgctaccagttcttcgacgagagcaagaactggtacgagagccaggccagctgcatgagccagaacgccagcctgctgaaggtgtacagcaaggaggaccaggacctgctgaagctggtgaagagctaccactggatgggcctggtgcacatccccaccaacggcagctggcagtgggaggacggcagcatcctgagccccaacctgctgaccatcatcgagatgcagaagggcgactgcgccctgtacgccagcagcttcaagggctacatcgagaactgcagcacccccaacacctacatctgcatgcagcggaccgtgagaagaaagagaagcggcagcggcgagggcagaggcagcctgctgacctgcggcgacgtggaggagaaccccggacccatgattcatctcggacatattctctttctcttgctcttgcctgtcgctgccgctcaaacaactcccggagaaagatcttctctccccgctttttatcccggaacatctggatcttgttctggatgtggatctttgtctctccctctcctcgctggactcgtcgcagctgatgctgtcgcttctctcttgattgtcggagctgtctttttgtgtaagagaggcagaaagaagctgctgtacatcttcaagcagcccttcatgagacccgtgcagaccacccaggaggaggacggctgcagctgcagattccccgaggaggaggagggcggctgcgagctg

SEQ ID NO: 77 - DNA, 1614 bp, synthetic construct
  source 1..1614: mol_type = other DNA
atgatccacctgggccacatcctgttcctgctgctgctgcccgtggccgctgcccagaccacccctggcgagcggagcagcctgcctgccttctaccctggcaccagcggcagctgcagcggctgcggcagcctgagcctgcccctgctggccggcctggtggccgccgacgccgtggccagcctgctgatcgtgggcgccgtgttcctgtgcgccaggcccaggcggagccctgcccaggaggacggcaaggtgtacatcaacatgcccggccggggctacttcctgggcaggctggtgcccaggggcaggggcgctgccgaggctgccacccggaagcagcggatcaccgagaccgagagcccctaccaggagctgcagggccagcggagcgacgtgtacagcgacctgaacacccagaggccctactacaagaggcggaaaaggtctgggagtggggctaccaatttctctctcctcaagcaagccggagacgttgaggaaaaccctggacccatgggctggatccggggacggaggagccggcacagctgggagatgagcgagttccacaactacaacctggacctgaagaagagcgacttcagcacccggtggcagaagcagcggtgccccgtggtgaagagcaagtgccgggagaacgccagccccttcttcttctgctgcttcatcgccgtggctatgggcatccggttcatcatcatggtggccatctggagcgccgtgttcctgaacagcctgttcaaccaggaggtgcagatccccctgaccgagagctactgcggcccctgccccaagaactggatctgctacaagaacaactgctaccagttcttcgacgagagcaagaactggtacgagagccaggccagctgcatgagccagaacgccagcctgctgaaggtgtacagcaaggaggaccaggacctgctgaagctggtgaagagctaccactggatgggcctggtgcacatccccaccaacggcagctggcagtgggaggacggcagcatcctgagccccaacctgctgaccatcatcgagatgcagaagggcgactgcgccctgtacgccagcagcttcaagggctacatcgagaactgcagcacccccaacacctacatctgcatgcagcggaccgtgagaagaaagagaagcggcagcggcgagggcagaggcagcctgctgacctgcggcgacgtggaggagaaccccggacctatggctctgcctgtgacagctctgctgctgcctctggctctgctgctgcacgccgctagacccgattataaggacgacgacgacaagcaaacaactcccggagaaagatcttctctccccgctttttatcccggaacatctggatcttgttctggatgtggatctttgtctctccctctcctcgctggactcgtcgcagctgatgctgtcgcttctctcttgattgtcggagctgtctttttgtgtaagagaggcagaaagaagctgctgtacatcttcaagcagcccttcatgagacccgtgcagaccacccaggaggaggacggctgcagctgcagattccccgaggaggaggagggcggctgcgagctg

SEQ ID NO: 78 - DNA, 1599 bp, synthetic construct
  source 1..1599: mol_type = other DNA
atgatccacctgggccacatcctgttcctgctgctgctgcccgtggccgctgcccagaccacccctggcgagcggagcagcctgcctgccttctaccctggcaccagcggcagctgcagcggctgcggcagcctgagcctgcccctgctggccggcctggtggccgccgacgccgtggccagcctgctgatcgtgggcgccgtgttcctgtgcgccaggcccaggcggagccctgcccaggaggacggcaaggtgtacatcaacatgcccggccggggctacttcctgggcaggctggtgcccaggggcaggggcgctgccgaggctgccacccggaagcagcggatcaccgagaccgagagcccctaccaggagctgcagggccagcggagcgacgtgtacagcgacctgaacacccagaggccctactacaagaggcggaaaaggtctgggagtggggctaccaatttctctctcctcaagcaagccggagacgttgaggaaaaccctggacccatgggctggatccggggacggaggagccggcacagctgggagatgagcgagttccacaactacaacctggacctgaagaagagcgacttcagcacccggtggcagaagcagcggtgccccgtggtgaagagcaagtgccgggagaacgccagccccttcttcttctgctgcttcatcgccgtggctatgggcatccggttcatcatcatggtggccatctggagcgccgtgttcctgaacagcctgttcaaccaggaggtgcagatccccctgaccgagagctactgcggcccctgccccaagaactggatctgctacaagaacaactgctaccagttcttcgacgagagcaagaactggtacgagagccaggccagctgcatgagccagaacgccagcctgctgaaggtgtacagcaaggaggaccaggacctgctgaagctggtgaagagctaccactggatgggcctggtgcacatccccaccaacggcagctggcagtgggaggacggcagcatcctgagccccaacctgctgaccatcatcgagatgcagaagggcgactgcgccctgtacgccagcagcttcaagggctacatcgagaactgcagcacccccaacacctacatctgcatgcagcggaccgtgagaagaaagagaagcggcagcggcgagggcagaggcagcctgctgacctgcggcgacgtggaggagaaccccggacccatgattcatctcggacatattctctttctcttgctcttgcctgtcgctgccgctcaaacaactcccggagaaagatcttctctccccgctttttatcccggaacatctggatcttgttctggatgtggatctttgtctctccctctcctcgctggactcgtcgcagctgatgctgtcgcttctctcttgattgtcggagctgtctttttgtgtcagaggcggaagtaccggagcaacaagggcgagagccccgtggagcctgccgagccctgccactacagctgtccccgggaggaggagggcagcaccatccccatccaggaggactaccggaagcccgagcctgcctgcagcccc

SEQ ID NO: 79 - DNA, 1632 bp, synthetic construct
  source 1..1632: mol_type = other DNA
atgatccacctgggccacatcctgttcctgctgctgctgcccgtggccgctgcccagaccacccctggcgagcggagcagcctgcctgccttctaccctggcaccagcggcagctgcagcggctgcggcagcctgagcctgcccctgctggccggcctggtggccgccgacgccgtggccagcctgctgatcgtgggcgccgtgttcctgtgcgccaggcccaggcggagccctgcccaggaggacggcaaggtgtacatcaacatgcccggccggggctacttcctgggcaggctggtgcccaggggcaggggcgctgccgaggctgccacccggaagcagcggatcaccgagaccgagagcccctaccaggagctgcagggccagcggagcgacgtgtacagcgacctgaacacccagaggccctactacaagaggcggaaaaggtctgggagtggggctaccaatttctctctcctcaagcaagccggagacgttgaggaaaaccctggacccatgggctggatccggggacggaggagccggcacagctgggagatgagcgagttccacaactacaacctggacctgaagaagagcgacttcagcacccggtggcagaagcagcggtgccccgtggtgaagagcaagtgccgggagaacgccagccccttcttcttctgctgcttcatcgccgtggctatgggcatccggttcatcatcatggtggccatctggagcgccgtgttcctgaacagcctgttcaaccaggaggtgcagatccccctgaccgagagctactgcggcccctgccccaagaactggatctgctacaagaacaactgctaccagttcttcgacgagagcaagaactggtacgagagccaggccagctgcatgagccagaacgccagcctgctgaaggtgtacagcaaggaggaccaggacctgctgaagctggtgaagagctaccactggatgggcctggtgcacatccccaccaacggcagctggcagtgggaggacggcagcatcctgagccccaacctgctgaccatcatcgagatgcagaagggcgactgcgccctgtacgccagcagcttcaagggctacatcgagaactgcagcacccccaacacctacatctgcatgcagcggaccgtgagaagaaagagaagcggcagcggcgagggcagaggcagcctgctgacctgcggcgacgtggaggagaaccccggacctatggctctgcctgtgacagctctgctgctgcctctggctctgctgctgcacgccgctagacccgattataaggacgacgacgacaagcaaacaactcccggagaaagatcttctctccccgctttttatcccggaacatctggatcttgttctggatgtggatctttgtctctccctctcctcgctggactcgtcgcagctgatgctgtcgcttctctcttgattgtcggagctgtctttttgtgtcagaggcggaagtaccggagcaacaagggcgagagccccgtggagcctgccgagccctgccactacagctgtccccgggaggaggagggcagcaccatccccatccaggaggactaccggaagcccgagcctgcctgcagcccc

SEQ ID NO: 80 - protein, 20 aa, synthetic construct
NAVPNLRGDLQVLAQKVART

SEQ ID NO: 81 - protein, 25 aa, synthetic construct
MGWLCSGLLFPVSCLVLLQVASSGN

SEQ ID NO: 82 - protein, 107 aa, Homo sapiens
IEVMYPPPYLDNEKSNGTIIHVKGKHLCPSPLFPGPSKPFWVLVVVGGVLACYSLLVTVAFIIFWVRSKRSRLLHSDYMNMTPRRPGPTRKHYQPYAPPRDFAAYRS

SEQ ID NO: 83 - protein, 112 aa, Homo sapiens
RVKFSRSADAPAYQQGQNQLYNELNLGRREEYDVLDKRRGRDPEMGGKPRRKNPQEGLYNELQKDKMAEAYSEIGMKGERRRGKGHDGLYQGLSTATKDTYDALHMQALPPR

SEQ ID NO: 84 - protein, 695 aa, synthetic construct
MGWSCIILFLVATATGVHSQIQLVQSGPELKKPGETVKISCKTSGYTFTDYSMHWVNQAPGKGLKWMGWINTETGEPTYTDDFKGRFAFSLETSASTAYLQINNLKNEDTATYFCARTAVYWGQGTTLTVSSGSTSGSGKPGSGEGSDIQMTQSPSSLSASLGERVSLTCRASQEISGSLSWLQQKPDGTIKRLIYAASTLNSGVPKRFSGRRSGSDYSLTISSLESEDFVDYYCLQYSSYPWSFGGGTKLEIKEPKSPDKTHTCPPCPSHTQPLGVFLFPPKPKDQLMISRTPEVTCVVVDVSQEDPEVQFNWYVDGVEVHNAKTKPREEQFNSTYRVVSVLTVLHQDWLNGKEYKCKVSNKGLPSSIEKTISKAKGQPREPQVYTLPPSQEEMTKNQVSLTCLVKGFYPSDIAVEWESNGQPENNYKTTPPVLDSDGSFFLYSRLTVDKSRWQEGNVFSCSVLHEALHNHYTQKSLSLSLGKFWVLVVVGGVLACYSLLVTVAFIIFWVARPRRSPAQEDGKVYINMPGRGGRLVPRGRGAAEAATRKQRITETESPYQELQGQRSDVYSDLNTQRPYYKRVKFSRSADAPAYQQGQNQLYNELNLGRREEYDVLDKRRGRDPEMGGKPQRRKNPQEGLYNELQKDKMAEAYSEIGMKGERRRGKGHDGLYQGLSTATKDTYDALHMQALPPR

SEQ ID NO: 85 - protein, 22 aa, synthetic construct
ARPRRSPAQEDGKVYINMPGRG

SEQ ID NO: 86 - protein, 49 aa, synthetic construct
GRLVPRGRGAAEAATRKQRITETESPYQELQGQRSDVYSDLNTQRPYYK

SEQ ID NO: 87 - protein, 360 aa, Homo sapiens
MEDFNMESDSFEDFWKGEDLSNYSYSSTLPPFLLDAAPCEPESLEINKYFVVIIYALVFLLSLLGNSLVMLVILYSRVGRSVTDVYLLNLALADLLFALTLPIWAASKVNGWIFGTFLCKVVSLLKEVNFYSGILLLACISVDRYLAIVHATRTLTQKRYLVKFICLSIWGLSLLLALPVLLFRRTVYSSNVSPACYEDMGNNTANWRMLLRILPQSFGFIVPLLIMLFCYGFTLRTLFKAHMGQKHRAMRVIFAVVLIFLLCWLPYNLVLLADTLMRTQVIQETCERRNHIDRALDATEILGILHSCLNPLIYAFIGQKFRHGLLKILAIHGLISKDSLPKDSRPSFVGSSSGHTSTTL

SEQ ID NO: 88 - DNA, 1080 bp, Homo sapiens
  source 1..1080: mol_type = other DNA
atggaggatttcaatatggagagcgactccttcgaggatttttggaagggcgaggacctgtctaactacagctatagctccacactgcccccttttctgctggatgccgccccttgtgagccagagtccctggagatcaacaagtacttcgtggtcatcatctatgccctggtgtttctgctgtctctgctgggcaatagcctggtcatgctggtcatcctgtactccagggtgggccgctctgtgaccgacgtgtatctgctgaatctggccctggccgatctgctgttcgcactgacactgccaatctgggcagcaagcaaggtgaacggctggatcttcggcacctttctgtgcaaggtggtgtctctgctgaaggaggtgaacttctacagcggcatcctgctgctggcctgtatctccgtggaccggtatctggccatcgtgcacgccaccaggacactgacccagaagcggtacctggtgaagttcatctgcctgagcatctggggactgtccctgctgctggccctgcctgtgctgctgtttaggcgcacagtgtactctagcaacgtgtctccagcctgttatgaggatatgggcaacaataccgccaattggaggatgctgctgcgcatcctgccacagagcttcggctttatcgtgcccctgctgatcatgctgttctgctacggctttacactgcggaccctgttcaaggcccacatgggccagaagcaccgggccatgagagtgatcttcgccgtggtgctgatctttctgctgtgctggctgccctataacctggtgctgctggccgacacactgatgcggacccaggtcatccaggagacatgcgagcggagaaaccacatcgacagagccctggatgccaccgagatcctgggcatcctgcactcctgtctgaatcctctgatctatgccttcatcggccagaagtttaggcacggcctgctgaagatcctggccatccacggcctgatctccaaggactctctgcccaaggatagccgcccttccttcgtgggctcctctagcggccacacctctaccacactg

SEQ ID NO: 89 - DNA, 8670 bp, synthetic construct
  source 1..8670: mol_type = other DNA
gatccggattagtccaatttgttaaagacaggatatcagtggtccaggctctagttttgactcaacaatatcaccagctgaagcctatagagtacgagccatagataaaataaaagattttatttagtctccagaaaaaggggggaatgaaagaccccacctgtaggtttggcaagctagcttaagtaacgccattttgcaaggcatggaaaaatacataactgagaatagagaagttcagatcaaggtcaggaacagatggaacagctgaatatgggccaaacaggatatctgtggtaagcagttcctgccccggctcagggccaagaacagatggaacagctgaatatgggccaaacaggatatctgtggtaagcagttcctgccccggctcagggccaagaacagatggtccccagatgcggtccagccctcagcagtttctagagaaccatcagatgtttccagggtgccccaaggacctgaaatgaccctgtgccttatttgaactaaccaatcagttcgcttctcgcttctgttcgcgcgcttctgctccccgagctcaataaaagagcccacaacccctcactcggggcgccagtcctccgattgactgagtcgcccgggtacccgtgtatccaataaaccctcttgcagttgcatccgacttgtggtctcgctgttccttgggagggtctcctctgagtgattgactacccgtcagcgggggtctttcacatgcagcatgtatcaaaattaatttggttttttttcttaagtatttacattaaatggccatagtacttaaagttacattggcttccttgaaataaacatggagtattcagaatgtgtcataaatatttctaattttaagatagtatctccattggctttctactttttcttttatttttttttgtcctctgtcttccatttgttgttgttgttgtttgtttgtttgtttgttggttggttggttaatttttttttaaagatcctacactatagttcaagctagactattagctactctgtaacccagggtgaccttgaagtcatgggtagcctgctgttttagccttcccacatctaagattacaggtatgagctatcatttttggtatattgattgattgattgattgatgtgtgtgtgtgtgattgtgtttgtgtgtgtgattgtgtatatgtgtgtatggttgtgtgtgattgtgtgtatgtatgtttgtgtgtgattgtgtgtgtgtgattgtgcatgtgtgtgtgtgtgattgtgtttatgtgtatgattgtgtgtgtgtgtgtgtgtgtgtgtgtgtgtgtgtgtgtgtgtgtgttgtgtatatatatttatggtagtgagaggcaacgctccggctcaggtgtcaggttggtttttgagacagagtctttcacttagcttggaattcactggccgtcgttttacaacgtcgtgactgggaaaaccctggcgttacccaacttaatcgccttgcagcacatccccctttcgccagctggcgtaatagcgaagaggcccgcaccgatcgcccttcccaacagttgcgcagcctgaatggcgaatggcgcctgatgcggtattttctccttacgcatctgtgcggtatttcacaccgcatatggtgcactctcagtacaatctgctctgatgccgcatagttaagccagccccgacacccgccaacacccgctgacgcgccctgacgggcttgtctgctcccggcatccgcttacagacaagctgtgaccgtctccgggagctgcatgtgtcagaggttttcaccgtcatcaccgaaacgcgcgagacgaaagggcctcgtgatacgcctatttttataggttaatgtcatgataataatggtttcttagacgtcaggtggcacttttcggggaaatgtgcgcggaacccctatttgtttatttttctaaatacattcaaatatgtatccgctcatgagacaataaccctgataaatgcttcaataatattgaaaaaggaagagtatgagtattcaacatttccgtgtcgcccttattcccttttttgcggcattttgccttcctgtttttgctcacccagaaacgctggtgaaagtaaaagatgctgaagatcagttgggtgcacgagtgggttacatcgaactggatctcaacagcggtaagatccttgagagttttcgccccgaagaacgttttccaatgatgagcacttttaaagttctgctatgtggcgcggtattatcccgtattgacgccgggcaagagcaactcggtcgccgcatacactattctcagaatgacttggttgagtactcaccagtcacagaaaagcatcttacggatggcatgacagtaagagaattatgcagtgctgccataaccatgagtgataacactgcggccaacttacttctgacaacgatcggaggaccgaaggagctaaccgcttttttgcacaacatgggggatcatgtaactcgccttgatcgttgggaaccggagctgaatgaagccataccaaacgacgagcgtgacaccacgatgcctgtagcaatggcaacaacgttgcgcaaactattaactggcgaactacttactctagcttcccggcaacaattaatagactggatggaggcggataaagttgcaggaccacttctgcgctcggcccttccggctggctggtttattgctgataaatctggagccggtgagcgtgggtctcgcggtatcattgcagcactggggccagatggtaagccctcccgtatcgtagttatctacacgacggggagtcaggcaactatggatgaacgaaatagacagatcgctgagataggtgcctcactgattaagcattggtaactgtcagaccaagtttactcatatatactttagattgatttaaaacttcatttttaatttaaaaggatctaggtgaagatcctttttgataatctcatgaccaaaatcccttaacgtgagttttcgttccactgagcgtcagaccccgtagaaaagatcaaaggatcttcttgagatcctttttttctgcgcgtaatctgctgcttgcaaacaaaaaaaccaccgctaccagcggtggtttgtttgccggatcaagagctaccaactctttttccgaaggtaactggcttcagcagagcgcagataccaaatactgttcttctagtgtagccgtagttaggccaccacttcaagaactctgtagcaccgcctacatacctcgctctgctaatcctgttaccagtggctgctgccagtggcgataagtcgtgtcttaccgggttggactcaagacgatagttaccggataaggcgcagcggtcgggctgaacggggggttcgtgcacacagcccagcttggagcgaacgacctacaccgaactgagatacctacagcgtgagctatgagaaagcgccacgcttcccgaagggagaaaggcggacaggtatccggtaagcggcagggtcggaacaggagagcgcacgagggagcttccagggggaaacgcctggtatctttatagtcctgtcgggtttcgccacctctgacttgagcgtcgatttttgtgatgctcgtcaggggggcggagcctatggaaaaacgccagcaacgcggcctttttacggttcctggccttttgctggccttttgctcacatgttctttcctgcgttatcccctgattctgtggataaccgtattaccgcctttgagtgagctgataccgctcgccgcagccgaacgaccgagcgcagcgagtcagtgagcgaggaagcggaagagcgcccaatacgcaaaccgcctctccccgcgcgttggccgattcattaatgcagctggcacgacaggtttcccgactggaaagcgggcagtgagcgcaacgcaattaatgtgagttagctcactcattaggcaccccaggctttacactttatgcttccggctcgtatgttgtgtggaattgtgagcggataacaatttcacacaggaaacagctatgaccatgattacgccaagctttgctcttaggagtttcctaatacatcccaaactcaaatatataaagcatttgacttgttctatgccctagggggcggggggaagctaagccagctttttttaacatttaaaatgttaattccattttaaatgcacagatgtttttatttcataagggtttcaatgtgcatgaatgctgcaatattcctgttaccaaagctagtataaataaaaatagataaacgtggaaattacttagagtttctgtcattaacgtttccttcctcagttgacaacataaatgcgctgctgagaagccagtttgcatctgtcaggatcaatttcccattatgccagtcatattaattactagtcaattagttgatttttatttttgacatatacatgtgaaagaccccacctgtaggtttggcaagctagcttaagtaacgccattttgcaaggcatggaaaaatacataactgagaatagaaaagttcagatcaaggtcaggaacagatggaacagctgaatatgggccaaacaggatatctgtggtaagcagttcctgccccggctcagggccaagaacagatggaacagctgaatatgggccaaacaggatatctgtggtaagcagttcctgccccggctcagggccaagaacagatggtccccagatgcggtccagccctcagcagtttctagagaaccatcagatgtttccagggtgccccaaggacctgaaatgaccctgtgccttatttgaactaaccaatcagttcgcttctcgcttctgttcgcgcgcttctgctccccgagctcaataaaagagcccacaacccctcactcggcgcgccagtcctccgattgactgagtcgcccgggtacccgtgtatccaataaaccctcttgcagttgcatccgacttgtggtctcgctgttccttgggagggtctcctctgagtgattgactacccgtcagcgggggtctttcatttgggggctcgtccgggatcgggagacccctgcccagggaccaccgacccaccaccgggaggtaagctggccagcaacttatctgtgtctgtccgattgtctagtgtctatgactgattttatgcgcctgcgtcggtactagttagctaactagctctgtatctggcggacccgtggtggaactgacgagttcggaacacccggccgcaaccctgggagacgtcccagggacttcgggggccgtttttgtggcccgacctgagtcctaaaatcccgatcgtttaggactctttggtgcaccccccttagaggagggatatgtggttctggtaggagacgagaacctaaaacagttcccgcctccgtctgaatttttgctttcggtttgggaccgaagccgcgccgcgcgtcttgtctgctgcagcatcgttctgtgttgtctctgtctgactgtgtttctgtatttgtctgaaaatatgggcccgggctagactgttaccactcccttaagtttgaccttaggtcactggaaagatgtcgagcggatcgctcacaaccagtcggtagatgtcaagaagagacgttgggttaccttctgctctgcagaatggccaacctttaacgtcggatggccgcgagacggcacctttaaccgagacctcatcacccaggttaagatcaaggtcttttcacctggcccgcatggacacccagaccaggtcccctacatcgtgacctgggaagccttggcttttgacccccctccctgggtcaagccctttgtacaccctaagcctccgcctcctcttcctccatccgccccgtctctcccccttgaacctcctcgttcgaccccgcctcgatcctccctttatccagccctcactccttctctaggcgcccccatatggccatatgagatcttatatggggcacccccgccccttgtaaacttccctgaccctgacatgacaagagttactaacagcccctctctccaagctcacttacaggctctctacttagtccagcacgaagtctggagacctctggcggcagcctaccaagaacaactggaccgaccggtggtacctcacccttaccgagtcggcgacacagtgtgggtccgccgacaccagactaagaacctagaacctcgctggaaaggaccttacacagtcctgctgaccacccccaccgccctcaaagtagacggcatcgcagcttggatacacgccgcccacgtgaaggctgccgaccccgggggtggaccatcctctagactgccatgatccacctgggccacatcctgttcctgctgctgctgcccgtggccgctgcccagaccacccctggcgagcggagcagcctgcctgccttctaccctggcaccagcggcagctgcagcggctgcggcagcctgagcctgcccctgctggccggcctggtggccgccgacgccgtggccagcctgctgatcgtgggcgccgtgttcctgtgcgccaggcccaggcggagccctgcccaggaggacggcaaggtgtacatcaacatgcccggccggggctacttcctgggcaggctggtgcccaggggcaggggcgctgccgaggctgccacccggaagcagcggatcaccgagaccgagagcccctaccaggagctgcagggccagcggagcgacgtgtacagcgacctgaacacccagaggccctactacaagaggcggaaaaggtctgggagtggggctaccaatttctctctcctcaagcaagccggagacgttgaggaaaaccctggacccatgggctggatccggggacggaggagccggcacagctgggagatgagcgagttccacaactacaacctggacctgaagaagagcgacttcagcacccggtggcagaagcagcggtgccccgtggtgaagagcaagtgccgggagaacgccagccccttcttcttctgctgcttcatcgccgtggctatgggcatccggttcatcatcatggtggccatctggagcgccgtgttcctgaacagcctgttcaaccaggaggtgcagatccccctgaccgagagctactgcggcccctgccccaagaactggatctgctacaagaacaactgctaccagttcttcgacgagagcaagaactggtacgagagccaggccagctgcatgagccagaacgccagcctgctgaaggtgtacagcaaggaggaccaggacctgctgaagctggtgaagagctaccactggatgggcctggtgcacatccccaccaacggcagctggcagtgggaggacggcagcatcctgagccccaacctgctgaccatcatcgagatgcagaagggcgactgcgccctgtacgccagcagcttcaagggctacatcgagaactgcagcacccccaacacctacatctgcatgcagcggacagtgcggagaaagagatccggatctggagagggaagaggaagcctgctgacctgcggcgacgtggaggagaacccaggacccatggaggatttcaatatggagagcgactccttcgaggatttttggaagggcgaggacctgtctaactacagctatagctccacactgcccccttttctgctggatgccgccccttgtgagccagagtccctggagatcaacaagtacttcgtggtcatcatctatgccctggtgtttctgctgtctctgctgggcaatagcctggtcatgctggtcatcctgtactccagggtgggccgctctgtgaccgacgtgtatctgctgaatctggccctggccgatctgctgttcgcactgacactgccaatctgggcagcaagcaaggtgaacggctggatcttcggcacctttctgtgcaaggtggtgtctctgctgaaggaggtgaacttctacagcggcatcctgctgctggcctgtatctccgtggaccggtatctggccatcgtgcacgccaccaggacactgacccagaagcggtacctggtgaagttcatctgcctgagcatctggggactgtccctgctgctggccctgcctgtgctgctgtttaggcgcacagtgtactctagcaacgtgtctccagcctgttatgaggatatgggcaacaataccgccaattggaggatgctgctgcgcatcctgccacagagcttcggctttatcgtgcccctgctgatcatgctgttctgctacggctttacactgcggaccctgttcaaggcccacatgggccagaagcaccgggccatgagagtgatcttcgccgtggtgctgatctttctgctgtgctggctgccctataacctggtgctgctggccgacacactgatgcggacccaggtcatccaggagacatgcgagcggagaaaccacatcgacagagccctggatgccaccgagatcctgggcatcctgcactcctgtctgaatcctctgatctatgccttcatcggccagaagtttaggcacggcctgctgaagatcctggccatccacggcctgatctccaaggactctctgcccaaggatagccgcccttccttcgtgggctcctctagcggccacacctctaccacactgtgacagccactcgag

SEQ ID NO: 90 - protein, 774 aa, synthetic construct
MIHLGHILFLLLLPVAAAQTTPGERSSLPAFYPGTSGSCSGCGSLSLPLLAGLVAADAVASLLIVGAVFLCARPRRSPAQEDGKVYINMPGRGYFLGRLVPRGRGAAEAATRKQRITETESPYQELQGQRSDVYSDLNTQRPYYKRRKRSGSGATNFSLLKQAGDVEENPGPMGWIRGRRSRHSWEMSEFHNYNLDLKKSDFSTRWQKQRCPVVKSKCRENASPFFFCCFIAVAMGIRFIIMVAIWSAVFLNSLFNQEVQIPLTESYCGPCPKNWICYKNNCYQFFDESKNWYESQASCMSQNASLLKVYSKEDQDLLKLVKSYHWMGLVHIPTNGSWQWEDGSILSPNLLTIIEMQKGDCALYASSFKGYIENCSTPNTYICMQRTVRRKRSGSGEGRGSLLTCGDVEENPGPMEDFNMESDSFEDFWKGEDLSNYSYSSTLPPFLLDAAPCEPESLEINKYFVVIIYALVFLLSLLGNSLVMLVILYSRVGRSVTDVYLLNLALADLLFALTLPIWAASKVNGWIFGTFLCKVVSLLKEVNFYSGILLLACISVDRYLAIVHATRTLTQKRYLVKFICLSIWGLSLLLALPVLLFRRTVYSSNVSPACYEDMGNNTANWRMLLRILPQSFGFIVPLLIMLFCYGFTLRTLFKAHMGQKHRAMRVIFAVVLIFLLCWLPYNLVLLADTLMRTQVIQETCERRNHIDRALDATEILGILHSCLNPLIYAFIGQKFRHGLLKILAIHGLISKDSLPKDSRPSFVGSSSGHTSTTL

SEQ ID NO: 91 - DNA, 2337 bp, synthetic construct
  source 1..2337: mol_type = other DNA
atgatccacctgggccacatcctgttcctgctgctgctgcccgtggccgctgcccagaccacccctggcgagcggagcagcctgcctgccttctaccctggcaccagcggcagctgcagcggctgcggcagcctgagcctgcccctgctggccggcctggtggccgccgacgccgtggccagcctgctgatcgtgggcgccgtgttcctgtgcgccaggcccaggcggagccctgcccaggaggacggcaaggtgtacatcaacatgcccggccggggctacttcctgggcaggctggtgcccaggggcaggggcgctgccgaggctgccacccggaagcagcggatcaccgagaccgagagcccctaccaggagctgcagggccagcggagcgacgtgtacagcgacctgaacacccagaggccctactacaagaggcggaaaaggtctgggagtggggctaccaatttctctctcctcaagcaagccggagacgttgaggaaaaccctggacccatgggctggatccggggacggaggagccggcacagctgggagatgagcgagttccacaactacaacctggacctgaagaagagcgacttcagcacccggtggcagaagcagcggtgccccgtggtgaagagcaagtgccgggagaacgccagccccttcttcttctgctgcttcatcgccgtggctatgggcatccggttcatcatcatggtggccatctggagcgccgtgttcctgaacagcctgttcaaccaggaggtgcagatccccctgaccgagagctactgcggcccctgccccaagaactggatctgctacaagaacaactgctaccagttcttcgacgagagcaagaactggtacgagagccaggccagctgcatgagccagaacgccagcctgctgaaggtgtacagcaaggaggaccaggacctgctgaagctggtgaagagctaccactggatgggcctggtgcacatccccaccaacggcagctggcagtgggaggacggcagcatcctgagccccaacctgctgaccatcatcgagatgcagaagggcgactgcgccctgtacgccagcagcttcaagggctacatcgagaactgcagcacccccaacacctacatctgcatgcagcggacagtgcggagaaagagatccggatctggagagggaagaggaagcctgctgacctgcggcgacgtggaggagaacccaggacccatggaggatttcaatatggagagcgactccttcgaggatttttggaagggcgaggacctgtctaactacagctatagctccacactgcccccttttctgctggatgccgccccttgtgagccagagtccctggagatcaacaagtacttcgtggtcatcatctatgccctggtgtttctgctgtctctgctgggcaatagcctggtcatgctggtcatcctgtactccagggtgggccgctctgtgaccgacgtgtatctgctgaatctggccctggccgatctgctgttcgcactgacactgccaatctgggcagcaagcaaggtgaacggctggatcttcggcacctttctgtgcaaggtggtgtctctgctgaaggaggtgaacttctacagcggcatcctgctgctggcctgtatctccgtggaccggtatctggccatcgtgcacgccaccaggacactgacccagaagcggtacctggtgaagttcatctgcctgagcatctggggactgtccctgctgctggccctgcctgtgctgctgtttaggcgcacagtgtactctagcaacgtgtctccagcctgttatgaggatatgggcaacaataccgccaattggaggatgctgctgcgcatcctgccacagagcttcggctttatcgtgcccctgctgatcatgctgttctgctacggctttacactgcggaccctgttcaaggcccacatgggccagaagcaccgggccatgagagtgatcttcgccgtggtgctgatctttctgctgtgctggctgccctataacctggtgctgctggccgacacactgatgcggacccaggtcatccaggagacatgcgagcggagaaaccacatcgacagagccctggatgccaccgagatcctgggcatcctgcactcctgtctgaatcctctgatctatgccttcatcggccagaagtttaggcacggcctgctgaagatcctggccatccacggcctgatctccaaggactctctgcccaaggatagccgcccttccttcgtgggctcctctagcggccacacctctaccacactgtgacagccactcgag

SEQ ID NO: 92 - protein, 329 aa, synthetic construct
MRVKFSRSADAPAYQQGQNQLYNELNLGRREEYDVLDKRRGRDPEMGGKPRRKNPQEGLYNELQKDKMAEAYSEIGMKGERRRGKGHDGLYQGLSTATKDTYDALHMQALPPRMGWIRGRRSRHSWEMSEFHNYNLDLKKSDFSTRWQKQRCPVVKSKCRENASPFFFCCFIAVAMGIRFIIMVAIWSAVFLNSLFNQEVQIPLTESYCGPCPKNWICYKNNCYQFFDESKNWYESQASCMSQNASLLKVYSKEDQDLLKLVKSYHWMGLVHIPTNGSWQWEDGSILSPNLLTIIEMQKGDCALYASSFKGYIENCSTPNTYICMQRTV

SEQ ID NO: 93 - DNA, 990 bp, synthetic construct
  source 1..990: mol_type = other DNA
atgagagtgaagttcagcaggagcgcagacgcccccgcgtaccagcagggccagaaccagctctataacgagctcaatctaggacgaagagaggagtacgatgttttggacaagagacgtggccgggaccctgagatggggggaaagccgagaaggaagaaccctcaggaaggcctgtacaatgaactgcagaaagataagatggcggaggcctacagtgagattgggatgaaaggcgagcgccggaggggcaaggggcacgatggcctttaccagggtctcagtacagccaccaaggacacctacgatgcattgcacatgcaggccctgccccctcgcatgggctggatccgcggccgcaggagccggcacagctgggagatgagcgagttccacaactacaacctggacctgaagaagagcgacttcagcacccggtggcagaagcagcggtgccccgtggtgaagagcaagtgccgggagaacgccagccccttcttcttctgctgcttcatcgccgtggctatgggcatccggtttataatcatggtggccatctggagcgccgtgttcctgaacagcctgttcaaccaggaggtgcagatccccctgaccgagagctactgcggcccctgccccaagaactggatctgctacaagaacaactgctaccagttcttcgacgagagcaagaactggtacgagagccaggccagctgcatgagccagaacgccagcctgctgaaggtgtacagcaaggaggaccaggacctgctgaagctggtgaagagctaccactggatgggcctggtgcacatccccaccaacggcagctggcagtgggaggacggcagcatcctgagccccaacctgctgaccatcatcgagatgcagaagggcgactgcgccctgtacgccagcagcttcaagggctacatcgagaactgcagcacccccaacacctacatctgcatgcagcggaccgtgtaa

SEQ ID NO: 94 - DNA, 1350 bp, synthetic construct
  source 1..1350: mol_type = other DNA
atgatccacctgggccacatcctgttcctgctgctgctgcccgtggccgctgcccagaccacccctggcgagcggagcagcctgcctgccttctaccctggcaccagcggcagctgcagcggctgcggcagcctgagcctgcccctgctggccggcctggtggccgccgacgccgtggccagcctgctgatcgtgggcgccgtgttcctgtgcgccaggcccaggcggagccctgcccaggaggacggcaaggtgtacatcaacatgcccggccggggcaggcggaaaaggtctgggagtggggctaccaatttctctctcctcaagcaagccggagacgttgaggaaaaccctggacccatgagagtgaagttcagcaggagcgcagacgcccccgcgtaccagcagggccagaaccagctctataacgagctcaatctaggacgaagagaggagtacgatgttttggacaagagacgtggccgggaccctgagatggggggaaagccgagaaggaagaaccctcaggaaggcctgtacaatgaactgcagaaagataagatggcggaggcctacagtgagattgggatgaaaggcgagcgccggaggggcaaggggcacgatggcctttaccagggtctcagtacagccaccaaggacacctacgatgcattgcacatgcaggccctgccccctcgcatgggctggatccgcggccgcaggagccggcacagctgggagatgagcgagttccacaactacaacctggacctgaagaagagcgacttcagcacccggtggcagaagcagcggtgccccgtggtgaagagcaagtgccgggagaacgccagccccttcttcttctgctgcttcatcgccgtggctatgggcatccggtttataatcatggtggccatctggagcgccgtgttcctgaacagcctgttcaaccaggaggtgcagatccccctgaccgagagctactgcggcccctgccccaagaactggatctgctacaagaacaactgctaccagttcttcgacgagagcaagaactggtacgagagccaggccagctgcatgagccagaacgccagcctgctgaaggtgtacagcaaggaggaccaggacctgctgaagctggtgaagagctaccactggatgggcctggtgcacatccccaccaacggcagctggcagtgggaggacggcagcatcctgagccccaacctgctgaccatcatcgagatgcagaagggcgactgcgccctgtacgccagcagcttcaagggctacatcgagaactgcagcacccccaacacctacatctgcatgcagcggaccgtgtaa

SEQ ID NO: 95 - protein, 135 aa, Homo sapiens; identical to SEQ ID NO: 16

SEQ ID NO: 96 - protein, 144 aa, Homo sapiens; identical to SEQ ID NO: 15

SEQ ID NO: 97 - protein, 127 aa, Homo sapiens
PLTESYCGPCPKNWICYKNNCYQFFDESKNWYESQASCMSQNASLLKVYSKEDQDLLKLVKSYHWMGLVHIPTNGSWQWEDGSILSPNLLTIIEMQKGDCALYASSFKGYIENCSTPNTYICMQRTV

SEQ ID NO: 98 - protein, 23 aa, Mus musculus
VVRVLAIALAIRFTLNTLMWLAI

SEQ ID NO: 99 - protein, 37 aa, Mus musculus
KISPMFVVRVLAIALAIRFTLNTLMWLAIFKETFQPV

SEQ ID NO: 100 - protein, 215 aa, Rattus exulans
MSKCHNYDLKPAKWDTSQEHQKQRSALPTSRPGENGIIRRRSSIEELKISPLFVVRVLVAAMTIRFTVITLTWLAVFITLLCNKEVSVSSREGYCGPCPNDWICHRNNCYQFFNENKAWNQSQASCLSQNSSLLKIYSKEEQDFLKLVKSYHWMGLVQSPANGSWQWEDGSSLSPNELTLVKTPSGTCAVYGSSFKAYTEDCSNPNTYICMKRAV

SEQ ID NO: 101 - protein, 23 aa, Rattus exulans
LFVVRVLVAAMTIRFTVITLTWL

SEQ ID NO: 102 - protein, 440 aa, synthetic construct
MALPVTALLLPLALLLHAARPDYKDDDDKLRPVQAQAQSDCSCSTVSPGVLAGIVMGDLVLTVLIALAVYFLGRLVPRGRGAAEAATRKQRITETESPYQELQGQRSDVYSDLNTQRPYYKRRKRSGSGEGRGSLLTCGDVEENPGPMIHLGHILFLLLLPVAAAQTTPGERSSLPAFYPGTSGSCSGCGSLSLPLLAGLVAADAVASLLIVGAVFLCARPRRSPAQEDGKVYINMPGRGRRKRSGSGATNFSLLKQAGDVEENPGPMKISPMFVVRVLAIALAIRFTLNTLMWLAIFKETFQPVLFNQEVQIPLTESYCGPCPKNWICYKNNCYQFFDESKNWYESQASCMSQNASLLKVYSKEDQDLLKLVKSYHWMGLVHIPTNGSWQWEDGSILSPNLLTIIEMQKGDCALYASSFKGYIENCSTPNTYICMQRTV

SEQ ID NO: 103 - DNA, 1320 bp, synthetic construct
  source 1..1320: mol_type = other DNA
atggctctgcctgtgacagctctgctgctgcctctggctctgctgctgcacgccgctagacccgattataaggacgacgacgacaagctgagacccgtgcaggcccaggcccagagcgactgcagctgcagcaccgtgagccccggcgtgctggccggcatcgtgatgggcgacctggtgctgaccgtgctcatcgcccttgccgtgtacttcctgggcagactggtccccaggggcagaggagctgccgaggccgctaccagaaagcagaggatcaccgagacagagagcccctaccaggagctgcagggccagagatccgacgtgtacagcgacctcaacacccagagaccctattacaagaggcggaagcgctccggctccggcgagggccgcggcagcctgctgacctgcggcgacgtggaagagaaccccggacccatgatccacctgggccacatcctgttcctgctgctgctgcccgtggccgctgcccaaacaacacccggcgagagatcctccttgcccgctttctatcccggaacatccggaagctgttccggatgtggatccctttctttgcctttgcttgctggattggtcgcagctgacgctgtcgcttccctccttattgtcggagctgtcttcctgtgcgccaggcccaggcggagccctgcccaggaggacggcaaggtgtacatcaacatgcccggccggggcaggcggaagcgctccgggagtggggctaccaatttctctctcctcaagcaagccggagacgttgaggaaaaccctggacccatgaaaatatctccaatgttcgttgttcgagtccttgctatagccttggcaattcgattcacccttaacacattgatgtggcttgccattttcaaagagacgtttcagccagtactgttcaaccaggaggtgcagatccccctgaccgagagctactgcggcccctgcccaaaaaattggatctgctacaagaacaactgctaccagttcttcgacgagagcaagaactggtacgagagccaggccagctgcatgagccagaacgccagcctgctgaaggtgtacagcaaggaggaccaggacctgctgaagctggtgaagagctaccactggatgggcctggtgcacatccccaccaacggcagctggcagtgggaggacggcagcatcctgagccccaacctgctgaccatcatcgagatgcagaagggcgactgcgccctgtacgccagcagcttcaagggctacatcgagaactgcagcacccccaacacctacatctgcatgcagcggaccgtg

SEQ ID NO: 104 - protein, 15 aa, Homo sapiens
EPKSCDKTHTCPPCP

SEQ ID NO: 105 - protein, 449 aa, synthetic construct
MIHLGHILFLLLLPVAAAQTTPGERSSLPAFYPGTSGSCSGCGSLSLPLLAGLVAADAVASLLIVGAVFLCARPRRSPAQEDGKVYINMPGRGRRKRSGSGATNFSLLKQAGDVEENPGPMRVKFSRSADAPAYQQGQNQLYNELNLGRREEYDVLDKRRGRDPEMGGKPRRKNPQEGLYNELQKDKMAEAYSEIGMKGERRRGKGHDGLYQGLSTATKDTYDALHMQALPPRMGWIRGRRSRHSWEMSEFHNYNLDLKKSDFSTRWQKQRCPVVKSKCRENASPFFFCCFIAVAMGIRFIIMVAIWSAVFLNSLFNQEVQIPLTESYCGPCPKNWICYKNNCYQFFDESKNWYESQASCMSQNASLLKVYSKEDQDLLKLVKSYHWMGLVHIPTNGSWQWEDGSILSPNLLTIIEMQKGDCALYASSFKGYIENCSTPNTYICMQRTV

SEQ ID NO: 106 - protein, 6 aa, Homo sapiens
MYPPPY

SEQ ID NO: 107 - protein, 4 aa, synthetic construct
GGGG

SEQ ID NO: 108 - protein, 5 aa, synthetic construct
GGGGG

SEQ ID NO: 109 - protein, 5 aa, synthetic construct
  REGION >5: note = The entire sequence of amino acids 1-5 can be repeated one to twenty times
GPPGS

SEQ ID NO: 110 - protein, 4 aa, synthetic construct
  REGION >4: note = The entire sequence of amino acids 1-4 can be repeated one or more times
  VARIANT 1: note = G residue can be repeated one or more times
  VARIANT 2: note = S residue can be repeated one or more times
GSGS

SEQ ID NO: 111 - protein, 4 aa, synthetic construct
  REGION >4: note = The entire sequence of amino acids 1-4 can be repeated one or more times
  VARIANT 1: note = S residue can be repeated one or more times
  VARIANT 2: note = G residue can be repeated one or more times
SGSG

SEQ ID NO: 112 - protein, 5 aa, synthetic construct
  REGION >5: note = The entire sequence of amino acids 1-5 can be repeated one or more times
EAAAK

SEQ ID NO: 113 - protein, 5 aa, synthetic construct
  REGION >5: note = The entire sequence of amino acids 1-5 can be repeated one or more times
GSGGG

SEQ ID NO: 114 - protein, 4 aa, synthetic construct
  REGION >4: note = The entire sequence of amino acids 1-4 can be repeated one or more times
SGGG

SEQ ID NO: 115 - protein, 5 aa, synthetic construct
  REGION >5: note = The entire sequence of amino acids 1-5 can be repeated one to twenty times
GGGGS